European Patent Specification EP 3 506 886 B1, published May 22, 2024. Title: Highly Concentrated Low Viscosity MASP-2 Inhibitory Antibody Formulations, Kits, and Methods. Applicant: Omeros Corporation Gregory A. Demopulos Kenneth M. Ferguson William Joseph Lambert John Steven Whitaker. The sequence listing filed with the application follows.

SEQUENCE LISTING (7 sequences)

SEQ ID NO: 1 - protein, 671 aa, Homo sapiens
TPLGPKWPEPVFGRLASPGFPGEYANDQERRWTLTAPPGYRLRLYFTHFDLELSHLCEYDFVKLSSGAKVLATLCGQESTDTERAPGKDTFYSLGSSLDITFRSDYSNEKPFTGFEAFYAAEDIDECQVAPGEAPTCDHHCHNHLGGFYCSCRAGYVLHRNKRTCSALCSGQVFTQRSGELSSPEYPRPYPKLSSCTYSISLEEGFSVILDFVESFDVETHPETLCPYDFLKIQTDREEHGPFCGKTLPHRIETKSNTVTITFVTDESGDHTGWKIHYTSTAQPCPYPMAPPNGHVSPVQAKYILKDSFSIFCETGYELLQGHLPLKSFTAVCQKDGSWDRPMPACSIVDCGPPDDLPSGRVEYITGPGVTTYKAVIQYSCEETFYTMKVNDGKYVCEADGFWTSSKGEKSLPVCEPVCGLSARTTGGRIYGGQKAKPGDFPWQVLILGGTTAAGALLYDNWVLTAAHAVYEQKHDASALDIRMGTLKRLSPHYTQAWSEAVFIHEGYTHDAGFDNDIALIKLNNKVVINSNITPICLPRKEAESFMRTDDIGTASGWGLTQRGFLARNLMYVDIPIVDHQKCTAAYEKPPYPRGSVTANMLCAGLESGGKDSCRGDSGGALVFLDSETERWFVGGIVSWGSMNCGEAGQYGVYTKVINYIPWIENIISDF

SEQ ID NO: 2 - protein, 118 aa, Artificial Sequence
  Synthetic
QVTLKESGPVLVKPTETLTLTCTVSGFSLSRGKMGVSWIRQPPGKALEWLAHIFSSDEKSYRTSLKSRLTISKDTSKNQVVLTMTNMDPVDTATYYCARIRRGGIDYWGQGTLVTVSS

SEQ ID NO: 3 - protein, 103 aa, Artificial Sequence
  Synthetic
QPVLTQPPSLSVSPGQTASITCSGEKLGDKYAYWYQQKPGQSPVLVMYQDKQRPSGIPERFSGSNSGNTATLTISGTQAMDEADYYCQAWDSSTAVFGGGTKL

SEQ ID NO: 4 - protein, 445 aa, Artificial Sequence
  Synthetic
QVTLKESGPVLVKPTETLTLTCTVSGFSLSRGKMGVSWIRQPPGKALEWLAHIFSSDEKSYRTSLKSRLTISKDTSKNQVVLTMTNMDPVDTATYYCARIRRGGIDYWGQGTLVTVSSASTKGPSVFPLAPCSRSTSESTAALGCLVKDYFPEPVTVSWNSGALTSGVHTFPAVLQSSGLYSLSSVVTVPSSSLGTKTYTCNVDHKPSNTKVDKRVESKYGPPCPPCPAPEFLGGPSVFLFPPKPKDTLMISRTPEVTCVVVDVSQEDPEVQFNWYVDGVEVHNAKTKPREEQFNSTYRVVSVLTVLHQDWLNGKEYKCKVSNKGLPSSIEKTISKAKGQPREPQVYTLPPSQEEMTKNQVSLTCLVKGFYPSDIAVEWESNGQPENNYKTTPPVLDSDGSFFLYSRLTVDKSRWQEGNVFSCSVMHEALHNHYTQKSLSLSLGK

SEQ ID NO: 5 - protein, 212 aa, Artificial Sequence
  Synthetic
QPVLTQPPSLSVSPGQTASITCSGEKLGDKYAYWYQQKPGQSPVLVMYQDKQRPSGIPERFSGSNSGNTATLTISGTQAMDEADYYCQAWDSSTAVFGGGTKLTVLGQPKAAPSVTLFPPSSEELQANKATLVCLISDFYPGAVTVAWKADSSPVKAGVETTTPSKQSNNKYAASSYLSLTPEQWKSHRSYSCQVTHEGSTVEKTVAPTECS

SEQ ID NO: 6 - DNA, 1395 bp, Artificial sequence
  Synthetic
atgatgtcctttgtctctctgctcctggttggcatcctattccatgccacccaggcccaggtcaccttgaaggagtctggtcctgtgctggtgaaacccacagagaccctcacgctgacctgcaccgtctctgggttctcactcagcaggggtaaaatgggtgtgagctggatccgtcagcccccagggaaggccctggagtggcttgcacacattttttcgagtgacgaaaaatcctacaggacatcgctgaagagcaggctcaccatctccaaggacacctccaaaaaccaggtggtccttacaatgaccaacatggaccctgtggacacagccacgtattactgtgcacggatacgacgtggaggaattgactactggggccagggaaccctggtcactgtctcctcagcctccaccaagggcccatccgtcttccccctggcgccctgctccaggagcacctccgagagcacagccgccctgggctgcctggtcaaggactacttccccgaaccggtgacggtgtcgtggaactcaggcgccctgaccagcggcgtgcacaccttcccggctgtcctacagtcctcaggactctactccctcagcagcgtggtgaccgtgccctccagcagcttgggcacgaagacctacacctgcaacgtagatcacaagcccagcaacaccaaggtggacaagagagttgagtccaaatatggtcccccatgcccaccatgcccagcacctgagttcctggggggaccatcagtcttcctgttccccccaaaacccaaggacactctcatgatctcccggacccctgaggtcacgtgcgtggtggtggacgtgagccaggaagaccccgaggtccagttcaactggtacgtggatggcgtggaggtgcataatgccaagacaaagccgcgggaggagcagttcaacagcacgtaccgtgtggtcagcgtcctcaccgtcctgcaccaggactggctgaacggcaaggagtacaagtgcaaggtctccaacaaaggcctcccgtcctccatcgagaaaaccatctccaaagccaaagggcagccccgagagccacaggtgtacaccctgcccccatcccaggaggagatgaccaagaaccaggtcagcctgacctgcctggtcaaaggcttctaccccagcgacatcgccgtggagtgggagagcaatgggcagccggagaacaactacaagaccacgcctcccgtgctggactccgacggctccttcttcctctacagcaggctaaccgtggacaagagcaggtggcaggaggggaatgtcttctcatgctccgtgatgcatgaggctctgcacaaccactacacacagaagagcctctccctgtctctcgggaaatga

SEQ ID NO: 7 - DNA, 696 bp, Artificial sequence
  Synthetic
  misc_feature (303)..(303): n is a, c, g, or t
atgatgtcctttgtctctctgctcctggttggcatcctattccatgccacccaggcccagccagtgctgactcagcccccctcactgtccgtgtccccaggacagacagccagcatcacctgctctggagagaaattgggggataaatatgcttactggtatcagcagaagccaggccagtcccctgtgttggtcatgtatcaagataaacagcggccctcagggatccctgagcgattctctggctccaactctgggaacacagccactctgaccatcagcgggacccaggctatggatgangctgactattactgtcaggcgtgggacagcagcactgcggtattcggcggagggaccaagctgaccgtcctaggccagcctaaggcggcgccctcggtcaccctgttcccgccctcctctgaggagcttcaagccaacaaggccacactggtgtgtctcataagtgacttctacccgggagccgtgacagtggcctggaaggcagatagcagccccgtcaaggcgggagtggagaccaccacaccctccaaacaaagcaacaacaagtacgcggccagcagctatctgagcctgacgcctgagcagtggaagtcccacagaagctacagctgccaggtcacgcatgaagggagcaccgtggagaagacagtggcccctacagaatgttcatag